European Patent Application EP 4 129 328 A1, published February 8, 2023. Title: Genetically modified Plasmodium parasite expressing Il-6 - Use to raise an immune response in a host against malaria at the pre-erythrocytic stage of development of the parasite. Applicant: INSTITUT PASTEUR. Application EPxxxxxxxx.x. The sequence listing filed with the application follows.

SEQUENCE LISTING (36 sequences)

SEQ ID NO: 1 - DNA, 636 bp, artificial sequence
  Synthetic sequence
atgaagttcctctctgcaagagacttccatccagttgccttcttgggactgatgctggtgacaaccacggccttccctacttcacaagtccggagaggagacttcacagaggataccactcccaacagacctgtctataccacttcacaagtcggaggcttaattacacatgttctctgggaaatcgtggaaatgagaaaagagttgtgcaatggcaattctgattgtatgaacaacgatgatgcacttgcagaaaacaatctgaaacttccagagatacaaagaaatgatggatgctaccaaactggatataatcaggaaatttgcctattgaaaatttcctctggtcttctggagtaccatagctacctggagtacatgaagaacaacttaaaagataacaagaaagacaaagccagagtccttcagagagatacagaaactctaattcatatcttcaaccaagaggtaaaagatttacataaaatagtccttcctaccccaatttccaatgctctcctaacagataagctggagtcacagaaggagtggctaaggaccaagaccatccaattcatcttgaaatcacttgaagaatttctaaaagtcactttgagatctactcggcaaacctag

SEQ ID NO: 2 - DNA, 564 bp, artificial sequence
  Synthetic sequence
tttccaacttcacaagtcagaagaggtgattttacagaagataccactccaaacagaccagtttacactacttctcaagttggtggtttgatcactcatgttttgtgggaaattgttgaaatgagaaaggaattgtgtaatggaaattctgattgtatgaacaacgatgatgctttggctgaaaataatttgaagttgccagagattcaaagaaatgatggatgttatcaaacaggatacaatcaagagatctgtttgctgaagatttcttctggattgttggagtatcattcttatttagaatacatgaaaaacaatttaaaggataacaagaaagacaaagctagagttttacagagagatactgaaactttgattcatattttcaaccaagaagttaaagatttgcataaaattgtccttccaacaccaatttcaaatgctttattgactgataaacttgaatctcagaaagaatggttgagaactaaaactattcagtttattttaaaatctttggaagaatttttgaaagttactttaagatctactagacaaacttaa

SEQ ID NO: 3 - DNA, 636 bp, artificial sequence
  Synthetic sequence
aactccttctccacaagcgccttcggtccagttgccttctccctggggctgctcctggtgttgcctgctgccttccctgccccagtacccccaggagaagattccaaagatgtagccgccccacacagacagccactcacctcttcagaacgaattgacaaacaaattcggtacatcctcgacggcatctcagccctgagaaaggagacatgtaacaagagtaacatgtgtgaaagcagcaaagaggcactggcagaaaacaacctgaaccttccaaagatggctgaaaaagatggatgcttccaatctggattcaatgaggagacttgcctggtgaaaatcatcactggtcttttggagtttgaggtatacctagagtacctccagaacagatttgagagtagtgaggaacaagccagagctgtgcagatgagtacaaaagtcctgatccagttcctgcagaaaaaggcaaagaatctagatgcaataaccacccctgacccaaccacaaatgccagcctgctgacgaagctgcaggcacagaaccagtggctgcaggacatgacaactcatctcattctgcgcagctttaaggagttcctgcagtccagcctgagggctcttcggcaaatgtag

SEQ ID NO: 4 - DNA, 636 bp, artificial sequence
  Synthetic sequence
aattcattttctacatctgcttttggtccagttgctttttcattaggtttattattagttttacctgctgcttttcctgctccagttccacctggagaagatagtaaagatgtagcagctccacatagacaacctttaacaagttcagaaagaatagataaacaaataagatatatattagatggtataagtgcattaagaaaagaaacatgtaataaatcaaatatgtgtgaaagttcaaaagaagcattagctgaaaataatttaaatttaccaaaaatggctgaaaaagatggatgttttcaatcaggttttaatgaagaaacatgtttagtaaaaataataacaggattattagaatttgaagtttatttagaatatttacaaaatagatttgaaagttcagaagaacaagcaagagctgtacaaatgagtacaaaagttttaatacaatttttacaaaagaaagcaaaaaatttagatgctataacaacaccagatcctacaacaaatgcatcattattaacaaaattacaagctcaaaatcaatggttacaagatatgacaacacatttaatattaagaagttttaaagaatttttacaatcatcattaagagcattaagacaaatgtaa

SEQ ID NO: 5 - DNA, 90 bp, artifical sequence
atgaaagatcatataaaaaatgtatgctttcggaaaactctactaatttcactactgcttattatattaaaatacacaaaatatgattat

SEQ ID NO: 6 - DNA, 62 bp, artifical sequence
atgtggtgggcctgtggtggctgctgctgctgctgctgctgctgtggcccatggtgtgggcc

SEQ ID NO: 7 - protein, 21 aa, artifical sequence
MWWRLWWLLLLLLLLWPMVWA

SEQ ID NO: 8 - DNA, 54 bp, artificial sequence
  Synthetic sequence
atgaagtgggtgaccttcatcagcctgctgttcctgttcagcagcgcctacagc

SEQ ID NO: 9 - protein, 18 aa, artificial sequence
  Synthetic sequence
MKWVTFISLLFLFSSAYS

SEQ ID NO: 10 - DNA, 1439 bp, artificial sequence
  Synthetic sequence
tggttaaatcgttttcacataaacgatgctatcaatttattaaagcatataataatataaaaaaaaagtatgatcaaaataaaacaatattataaatgttcttaaacatcaaaaaatggaatatatacattaaaaatgtgcacatcttttaagtgttcattagcatatatcatttttcgtatgatctttaaatctagaagtcctcctacacatgtgaatgtatatgtatataattttttaacgatgtaacagtgttgtatatattattgaagatatacattatttatgttaaaaaatcatgtaaacaaaattataggaataaactaattttgaatcatttatttgcttaaaaattaaccacattatatttaataaatataaaataaaaatatgccacatccattctatactatttattggtacatcgacattcgccataaaatatttcatagagttgcattatcgtcaaaagtgtataaaattataaaatagagcaacataaaatggataataatggtgaaactaaaaataataaaattaaagttgggtaaataaaaacacaacataaaggatcaaggtattatttttttaaattttttttatgaaaaactattagaacaatttaaaataatgcatattatgctttatttgtacaatataattaaaataaaacgaataacgatgtgattattcaatatgcagattaataatatatacacatgtaaatgtatatatacttcttcattgtcaaattccttaggcatatgtagcatatatggtttttgacggttctttaaaaatatacaactgtaatccctaataaatgaatgcagttgaaatcgaacaaatccatatgcttccgtatcgatttaaccatttaggtagtgatctatgatcgatctacatgtgaagaaaattggcatcttttaaaaactctttcataatggtttatgagttctttagatcatatattatttaaacaaaaaataaaataaatcacctatttttttatattcgataaagcgtgcaaacaaatttgcatgtatgtattctattatcgttggttttttttacaccaccttttttttatttataatgtttttcaccacaaagcaactatatataaaaaacacactaaaaatatataattaaattaaaaaataataataaagaaaataaaaaataaaaaataaaaagcatatgtattatacatgcatgtatattcccctgcatatgtatgttttcagttcagattaagaacaaaaaaatacagataattaagcatttatttgttacgtttatacatgtcaataccaaaaatatatatgtgcctacacatgttacatataagtagatacatataaatatatcggagtaatattcttcttctttcatttttcacttctattataatcattttacttttttacacataaaaa

SEQ ID NO: 11 - DNA, 1501 bp, artificial sequence
  Synthetic sequence
tgtttaataccaatacttagaaataaataaatatgtagatatttagatatataatacttttttttcagtgtataaaaaatttattaaacatgtaaataaatatatatacacacatatatatatatatattattattattatatgtgaacaatatttcatatatataatgcttgattaatataaaaaaaagaaatttttatttttttaaattatatccttacaataaataaggctctatcaaattttataaaacatgtaagaataaaaaataaaaaaaaatatacgtaatatatatatatatatatatatatatatatatatttatttatttatttatttatttttattttttctttcctatgtagatatatgcaacccactctacaagacactcgaaaagtaacaaaaaagaaaaagagacaaatgagtaacatacatacatgtatatttatcaacatgtttgcttcgatatattcacacattttttttcttattcttttttttttttttgggtatatatgtgtggatctaacgtgataaatattaggcgaaaaaaaaaaaaaaaaaaatataggaacattttaatatcaccattagaacaatcgacacatttatatataacgtcgatgatgaaagctgatcattttttaaccatcttataatgtattcttttcattatgtttaaataaaaaattatatatatattattaatttattcccactgcaataatattaaaagacacataaaataattatattaaaacaatgtggttctttattttttttttaatatttttcacatataaatatataaatatataaataaataaataaataaatatatatatatatatatatgtaaggtatttagaatttttttttttttttttttttataagaccatttaagtggcgcatttttcccttaattttttcttatatttttatactatcaaaattaatatttttggtttaaatacacagaaagaaaaaagaaaaatatataaatagaacatatattaataaattatttcaaataactatacatatatatatatatatatatattatttataatttttagaaatattagcttattatatattactccatttgaaccttattttaataagaataaaaattgtaaaaaaatattttattattattttattttttttctcataaatacaaggtcaaatactttcttgtttattttttcgcagtatcaaaaaatacgaataaaatgagaataaatttaatttcacgtacttttaaatatttttatttttcaaaatttattccaatattggtattaaattcatttgtaatatattttattttacataataataataaaataaatatatacatatatatatgtatatactttttatatatttatatgattattttgttatatcaacaaatctataaaacacattatttcttaagaccttaatatgcacttatatacgatgtattcttttttaaattattaaaaa

SEQ ID NO: 12 - DNA, 1501 bp, artificial sequence
  Synthetic sequence
tcttttattctaaagatacataaattcgttttattaattaataaacaaagttttccttattcttattagctaatattgaaaaaatgaaattgtgtataaaaaaaaaataaatatatacatagaaacatatatatatgtagaatacaaccaatatgtgtatacacacataaatataaatatatatatatatatatatttatatatatgcatatatttatttattttatttatttttttttttttgtgcttgttttaaaaattttccttttagaaatttattcagttctgttctaaataaaacattataattcatcaataataacttttttacttaaatataaaaaaaaggacgatagacaaacaaaaataaaataatataaaataaaatacataataatataatgttgaaaatattaccaataatatttttttacaaattttgaatattaaccataaggaatataattatttatcataccaattaaacctatattatatgtgtaaattgaaaagaatagaacgttacacaaatttataagtatatatattaacataaaatatatatatttcttttatataaatagataaaagttatattaataaataatttatttatacattattttattattaaaatattttaagtattttattttattatatttttttttgagttgtcgataggttcgatcaataatatggaaagttatatgtttcttctattatagatactattagaaaatatattccacatgtgtacatatatatatatatatatatatatacatatacgcatgtaaattcaaaagaaaatcttaaaaaagaaaaacatattaatgttaataatatttatatataattataatacattgtgctatttttgttatcaatttggtgaacaaacacaatttatgagaacagaacaatatttacaaaattggccttctatagaatagttataagtacagaaatattttattttcaaaaaatattaaattataatacacaagaaaaaatatattcgacatatatatatatatatatattaatttcttaaatcgaaattttattttaaaatatatatcaaaattatatgttttttttcttagggaaaaatatatcccatctattattaaacgtttatcgttttatggacaagctactgaaaacgtaataaatatatatatatatatatatatatatatatacctaccaaggtttatatacttttttgatatttatatatttaatcttaaattctgttaataaattaaatattttaattaaattattcttaaatatgaaaatgtattgatcttatttagcttatcattactgtactttattcatatatatgatattaatattaattttatgataatttaaatcatacatcttaagataaacaaaaaaaaaaaaatttaccaaatacatggttaataaatatacaaaaaaatgttataaaaaacatattgtgtgtttatataatgatatatttttt

SEQ ID NO: 13 - DNA, 1833 bp, artificial sequence
  Synthetic sequence
ccatggccaacacttgtcactactttcgcgtatggtcttcaatgctttgcgagatacccagatcatatgaaacagcatgactttttcaagagtgccatgcccgaaggttatgtacaggaaagaactatatttttcaaagatgacgggaactacaagacacgtgctgaagtcaagtttgaaggtgatacccttgttaatagaatcgagttaaaaggtattgattttaaagaagatggaaacattcttggacacaaattggaatacaactataactcacacaatgtatacatcatggcagacaaacaaaagaatggaatcaaagttaacttcaaaattagacacaacattgaagatggaagcgttcaactagcagaccattatcaacaaaatactccaattggcgatggccctgtccttttaccagacaaccattacctgtccacacaatctgccctttcgaaagatcccaacgaaaagagagaccacatggtccttcttgagtttgtaacagctgctgggattacacatggcatggatgaactatacaaaggttcgggagagggcagaggatccctgctaacatgcggtgatgtcgaggagaatcctggcccaatggttggttcgctaaactgcatcgtcgctgtgtcccagaacatgggcatcggcaagaacggggacctgccctggccaccgctcaggaacgaatttagatatttccagagaatgaccacaacctcttcagtagaaggtaaacagaatctggtgattatgggtaagaagacctggttctccattcctgagaagaatcgacctttaaagggtagaattaatttagttctcagcagagaactcaaggaacctccacaaggagctcattttctttccagaagtctagatgatgccttaaaacttactgaacaaccagaattagcaaataaagtagacatggtctggatagttggtggcagttctgtttataaggaagccatgaatcacccaggccatcttaaactatttgtgacaaggatcatgcaagactttgaaagtgacacgttttttccagaaattgatttggagaaatataaacttctgccagaatacccaggtgttctctctgatgtccaggaggagaaaggcattaagtacaaatttgaagtatatgagaagaatgattaaattattaatatatatgaatatatatacatcgttgtatgcgtaatatacgtgtaactgttttttttaatttttatattaacttttccttatacattttaatgccattaactaataatattttacttgaaaaaattctaaatttttataactctaatataaaatctgtgaataataaaaaattagcataaagtacgaattaaacatcgaatatttgttttaaaggggcacacattatgtgcatataattttattctttgaatttaattttttgcttataattagattaaattaatataatttttttattgaaaataaaaacttattttaaaaaattaacaaatggaagttaatgaaaaatacgaaaaaagtaaagggttaattcttatatggtcatataaaaaaacaaatgaaataatgtaaacagttattcattttttaagggtataaaataagcttataaataatgttagcatattaaaaacagtgatataagtatgtgtaaatatgaaagaatataataatggatagttaaaaaaatatattttaaagggaatattgacaaattatatactgaagcactaaagaaaatatcatctttgtatattatagcttcacatttccaagcaaatggtgccacaaatacattcttctctctcc

SEQ ID NO: 14 - DNA, 2927 bp, artificial sequence
  Synthetic sequence
tggttaaatcgttttcacataaacgatgctatcaatttattaaagcatataataatataaaaaaaaagtatgatcaaaataaaacaatattataaatgttcttaaacatcaaaaaatggaatatatacattaaaaatgtgcacatcttttaagtgttcattagcatatatcatttttcgtatgatctttaaatctagaagtcctcctacacatgtgaatgtatatgtatataattttttaacgatgtaacagtgttgtatatattattgaagatatacattatttatgttaaaaaatcatgtaaacaaaattataggaataaactaattttgaatcatttatttgcttaaaaattaaccacattatatttaataaatataaaataaaaatatgccacatccattctatactatttattggtacatcgacattcgccataaaatatttcatagagttgcattatcgtcaaaagtgtataaaattataaaatagagcaacataaaatggataataatggtgaaactaaaaataataaaattaaagttgggtaaataaaaacacaacataaaggatcaaggtattatttttttaaattttttttatgaaaaactattagaacaatttaaaataatgcatattatgctttatttgtacaatataattaaaataaaacgaataacgatgtgattattcaatatgcagattaataatatatacacatgtaaatgtatatatacttcttcattgtcaaattccttaggcatatgtagcatatatggtttttgacggttctttaaaaatatacaactgtaatccctaataaatgaatgcagttgaaatcgaacaaatccatatgcttccgtatcgatttaaccatttaggtagtgatctatgatcgatctacatgtgaagaaaattggcatcttttaaaaactctttcataatggtttatgagttctttagatcatatattatttaaacaaaaaataaaataaatcacctatttttttatattcgataaagcgtgcaaacaaatttgcatgtatgtattctattatcgttggttttttttacaccaccttttttttatttataatgtttttcaccacaaagcaactatatataaaaaacacactaaaaatatataattaaattaaaaaataataataaagaaaataaaaaataaaaaataaaaagcatatgtattatacatgcatgtatattcccctgcatatgtatgttttcagttcagattaagaacaaaaaaatacagataattaagcatttatttgttacgtttatacatgtcaataccaaaaatatatatgtgcctacacatgttacatataagtagatacatataaatatatcggagtaatattcttcttctttcatttttcacttctattataatcattttacttttttacacataaaaaatgaaagatcatataaaaaatgtatgctttcggaaaactctactaatttcactactgcttattatattaaaatacacaaaatatgattattttccaacttcacaagtcagaagaggtgattttacagaagataccactccaaacagaccagtttacactacttctcaagttggtggtttgatcactcatgttttgtgggaaattgttgaaatgagaaaggaattgtgtaatggaaattctgattgtatgaacaacgatgatgctttggctgaaaataatttgaagttgccagagattcaaagaaatgatggatgttatcaaacaggatacaatcaagagatctgtttgctgaagatttcttctggattgttggagtatcattcttatttagaatacatgaaaaacaatttaaaggataacaagaaagacaaagctagagttttacagagagatactgaaactttgattcatattttcaaccaagaagttaaagatttgcataaaattgtccttccaacaccaatttcaaatgctttattgactgataaacttgaatctcagaaagaatggttgagaactaaaactattcagtttattttaaaatctttggaagaatttttgaaagttactttaagatctactagacaaacttaactcgaggaattctcgtttttcttatttatatatttataccaattgattgtatttataactgtaaaaatgtgtatgttgtgtgcatatttttttttgtgcatgcacatgcatgtaaatagctaaaattatgaacattttattttttgttcagaaaaaaaaaactttacacacataaaatggctagtatgaatagccatattttatataaattaaatcctatgaatttatgaccatattaaaaatttagatatttatggaacataatatgtttgaaacaataagacaaaattattattattattattatttttactgttataattatgttgtctcttcaatgattcataaatagttggacttgatttttaaaatgtttataatatgattagcatagttaaataaaaaaagttgaaaaattaaaaaaaaacatataaacacaaatgatgttttttccttcaatttcgatatcatatagcaatcgtattagcaggtaaatgagcaaggttaataaaaaaatggtaaaaaaaaaaaaattggggaaaaataaacaaggtgttctttatctacactttggctttacaatgtataatttatatgcatacaaaaaaattttgataaaattgtaaaaaggtgaataaaataacattgtaacagtagtagatagtaaagggaaggtgttgctcaaatagtgtcgaaacaaaactggcataaagaaaaattgatattgagcagaggatatgcgcataatggtattttgtttgtttgtttgttttctcattttttgagacagctcaattctttatgtccacaacatcatcggacttttcttcttca

SEQ ID NO: 15 - DNA, 2093 bp, artificial sequence
  Synthetic sequence
tggttaaatcgttttcacataaacgatgctatcaatttattaaagcatataataatataaaaaaaaagtatgatcaaaataaaacaatattataaatgttcttaaacatcaaaaaatggaatatatacattaaaaatgtgcacatcttttaagtgttcattagcatatatcatttttcgtatgatctttaaatctagaagtcctcctacacatgtgaatgtatatgtatataattttttaacgatgtaacagtgttgtatatattattgaagatatacattatttatgttaaaaaatcatgtaaacaaaattataggaataaactaattttgaatcatttatttgcttaaaaattaaccacattatatttaataaatataaaataaaaatatgccacatccattctatactatttattggtacatcgacattcgccataaaatatttcatagagttgcattatcgtcaaaagtgtataaaattataaaatagagcaacataaaatggataataatggtgaaactaaaaataataaaattaaagttgggtaaataaaaacacaacataaaggatcaaggtattatttttttaaattttttttatgaaaaactattagaacaatttaaaataatgcatattatgctttatttgtacaatataattaaaataaaacgaataacgatgtgattattcaatatgcagattaataatatatacacatgtaaatgtatatatacttcttcattgtcaaattccttaggcatatgtagcatatatggtttttgacggttctttaaaaatatacaactgtaatccctaataaatgaatgcagttgaaatcgaacaaatccatatgcttccgtatcgatttaaccatttaggtagtgatctatgatcgatctacatgtgaagaaaattggcatcttttaaaaactctttcataatggtttatgagttctttagatcatatattatttaaacaaaaaataaaataaatcacctatttttttatattcgataaagcgtgcaaacaaatttgcatgtatgtattctattatcgttggttttttttacaccaccttttttttatttataatgtttttcaccacaaagcaactatatataaaaaacacactaaaaatatataattaaattaaaaaataataataaagaaaataaaaaataaaaaataaaaagcatatgtattatacatgcatgtatattcccctgcatatgtatgttttcagttcagattaagaacaaaaaaatacagataattaagcatttatttgttacgtttatacatgtcaataccaaaaatatatatgtgcctacacatgttacatataagtagatacatataaatatatcggagtaatattcttcttctttcatttttcacttctattataatcattttacttttttacacataaaaaatgaaagatcatataaaaaatgtatgctttcggaaaactctactaatttcactactgcttattatattaaaatacacaaaatatgattattttccaacttcacaagtcagaagaggtgattttacagaagataccactccaaacagaccagtttacactacttctcaagttggtggtttgatcactcatgttttgtgggaaattgttgaaatgagaaaggaattgtgtaatggaaattctgattgtatgaacaacgatgatgctttggctgaaaataatttgaagttgccagagattcaaagaaatgatggatgttatcaaacaggatacaatcaagagatctgtttgctgaagatttcttctggattgttggagtatcattcttatttagaatacatgaaaaacaatttaaaggataacaagaaagacaaagctagagttttacagagagatactgaaactttgattcatattttcaaccaagaagttaaagatttgcataaaattgtccttccaacaccaatttcaaatgctttattgactgataaacttgaatctcagaaagaatggttgagaactaaaactattcagtttattttaaaatctttggaagaatttttgaaagttactttaagatctactagacaaacttaa

SEQ ID NO: 16 - DNA, 549 bp, artificial sequence
  Synthetic sequence
ccatggccaacacttgtcactactttcgcgtatggtcttcaatgctttgcgagatacccagatcatatgaaacagcatgactttttcaagagtgccatgcccgaaggttatgtacaggaaagaactatatttttcaaagatgacgggaactacaagacacgtgctgaagtcaagtttgaaggtgatacccttgttaatagaatcgagttaaaaggtattgattttaaagaagatggaaacattcttggacacaaattggaatacaactataactcacacaatgtatacatcatggcagacaaacaaaagaatggaatcaaagttaacttcaaaattagacacaacattgaagatggaagcgttcaactagcagaccattatcaacaaaatactccaattggcgatggccctgtccttttaccagacaaccattacctgtccacacaatctgccctttcgaaagatcccaacgaaaagagagaccacatggtccttcttgagtttgtaacagctgctgggattacacatggcatggatgaactatacaaa

SEQ ID NO: 17 - DNA, 63 bp, artificial sequence
  Synthetic sequence
ggttcgggagagggcagaggatccctgctaacatgcggtgatgtcgaggagaatcctggccca

SEQ ID NO: 18 - DNA, 564 bp, artificial sequence
  Synthetic sequence
atggttggttcgctaaactgcatcgtcgctgtgtcccagaacatgggcatcggcaagaacggggacctgccctggccaccgctcaggaacgaatttagatatttccagagaatgaccacaacctcttcagtagaaggtaaacagaatctggtgattatgggtaagaagacctggttctccattcctgagaagaatcgacctttaaagggtagaattaatttagttctcagcagagaactcaaggaacctccacaaggagctcattttctttccagaagtctagatgatgccttaaaacttactgaacaaccagaattagcaaataaagtagacatggtctggatagttggtggcagttctgtttataaggaagccatgaatcacccaggccatcttaaactatttgtgacaaggatcatgcaagactttgaaagtgacacgttttttccagaaattgatttggagaaatataaacttctgccagaatacccaggtgttctctctgatgtccaggaggagaaaggcattaagtacaaatttgaagtatatgagaagaatgattaa

SEQ ID NO: 19 - DNA, 657 bp, artificial sequence
  Synthetic sequence
attattaatatatatgaatatatatacatcgttgtatgcgtaatatacgtgtaactgttttttttaatttttatattaacttttccttatacattttaatgccattaactaataatattttacttgaaaaaattctaaatttttataactctaatataaaatctgtgaataataaaaaattagcataaagtacgaattaaacatcgaatatttgttttaaaggggcacacattatgtgcatataattttattctttgaatttaattttttgcttataattagattaaattaatataatttttttattgaaaataaaaacttattttaaaaaattaacaaatggaagttaatgaaaaatacgaaaaaagtaaagggttaattcttatatggtcatataaaaaaacaaatgaaataatgtaaacagttattcattttttaagggtataaaataagcttataaataatgttagcatattaaaaacagtgatataagtatgtgtaaatatgaaagaatataataatggatagttaaaaaaatatattttaaagggaatattgacaaattatatactgaagcactaaagaaaatatcatctttgtatattatagcttcacatttccaagcaaatggtgccacaaatacattcttctctctcc

SEQ ID NO: 20 - DNA, 822 bp, artificial sequence
  Synthetic sequence
tcgtttttcttatttatatatttataccaattgattgtatttataactgtaaaaatgtgtatgttgtgtgcatatttttttttgtgcatgcacatgcatgtaaatagctaaaattatgaacattttattttttgttcagaaaaaaaaaactttacacacataaaatggctagtatgaatagccatattttatataaattaaatcctatgaatttatgaccatattaaaaatttagatatttatggaacataatatgtttgaaacaataagacaaaattattattattattattatttttactgttataattatgttgtctcttcaatgattcataaatagttggacttgatttttaaaatgtttataatatgattagcatagttaaataaaaaaagttgaaaaattaaaaaaaaacatataaacacaaatgatgttttttccttcaatttcgatatcatatagcaatcgtattagcaggtaaatgagcaaggttaataaaaaaatggtaaaaaaaaaaaaattggggaaaaataaacaaggtgttctttatctacactttggctttacaatgtataatttatatgcatacaaaaaaattttgataaaattgtaaaaaggtgaataaaataacattgtaacagtagtagatagtaaagggaaggtgttgctcaaatagtgtcgaaacaaaactggcataaagaaaaattgatattgagcagaggatatgcgcataatggtattttgtttgtttgtttgttttctcattttttgagacagctcaattctttatgtccacaacatcatcggacttttcttcttca

SEQ ID NO: 21 - DNA, 41 bp, artificial sequence
  Synthetic sequence
ccgcctaggaaaatgagtaaaggagaagaacttttcactgg

SEQ ID NO: 22 - DNA, 39 bp, artificial sequence
  Synthetic sequence
cgcaattgtgaaattaataaaataaaatacatatccctc

SEQ ID NO: 23 - DNA, 27 bp, artificial sequence
  Synthetic sequence
tgcatgcacaaaaaaaaatatgcacac

SEQ ID NO: 24 - DNA, 37 bp, artificial sequence
  Synthetic sequence
ccggaattcttaaacacagtagtatctgtcaccaaag

SEQ ID NO: 25 - DNA, 41 bp, artificial sequence
  Synthetic sequence
acaaaatatgattattttccaacttcacaagtcagaagagg

SEQ ID NO: 26 - DNA, 35 bp, artificial sequence
  Synthetic sequence
ccgcctaggtataaaatttttatttatttataagc

SEQ ID NO: 27 - DNA, 24 bp, artificial sequence
  Synthetic sequence
attaatcttgaacgaggaatggct

SEQ ID NO: 28 - DNA, 19 bp, artificial sequence
  Synthetic sequence
tcaatcggtaggagcgacg

SEQ ID NO: 29 - DNA, 20 bp, artificial sequence
  Synthetic sequence
gccaaatgctaaacctaatg

SEQ ID NO: 30 - DNA, 20 bp, artificial sequence
  Synthetic sequence
tgggtttgtattgtatgcac

SEQ ID NO: 31 - DNA, 17 bp, artificial sequence
  Synthetic sequence
tgcagctaatcaaactc

SEQ ID NO: 32 - DNA, 20 bp, artificial sequence
  Synthetic sequence
acttcaatttgtggaacacc

SEQ ID NO: 33 - DNA, 20 bp, artificial sequence
  Synthetic sequence
ctggtgaaaaggacctctcg

SEQ ID NO: 34 - DNA, 26 bp, artificial sequence
  Synthetic sequence
tgaagtactcattatagtcaagggca

SEQ ID NO: 35 - DNA, 25 bp, artificial sequence
  Synthetic sequence
aaagaaatgatggatgctaccaaac

SEQ ID NO: 36 - DNA, 33 bp, artificial sequence
  Synthetic sequence
cttgttatcttttaagttgttcttcatgtactc